European Patent Application EP 4 406 972 A1, published July 31, 2024. Title: GFRAL antagonist antibody with improved affinity and use thereof. Applicant: Daegu Gyeongbuk Institute of Science and Technology. The sequence listing filed with the application follows.

SEQUENCE LISTING (10 sequences)

SEQ ID NO: 1 - protein, 8 aa, synthetic construct
GFTFSSYG

SEQ ID NO: 2 - protein, 8 aa, synthetic construct
ISFDGSNK

SEQ ID NO: 3 - protein, 21 aa, synthetic construct
CAKVTSGGDFLSGNYYYYMDV

SEQ ID NO: 4 - protein, 6 aa, synthetic construct
SLRDYY

SEQ ID NO: 5 - skipped

SEQ ID NO: 6 - protein, 11 aa, synthetic construct
NSRGSSGNQWV

SEQ ID NO: 7 - protein, 8 aa, synthetic construct
ISYDGSNK

SEQ ID NO: 8 - protein, 21 aa, synthetic construct
CAKVTSGGDFWSGDYYWYMDV

SEQ ID NO: 9 - protein, 6 aa, synthetic construct
SLRDNK

SEQ ID NO: 10 - skipped